European Patent Application EP 4 154 907 A1, published March 29, 2023. Title: INFLUENZA VIRUS VACCINES AND USES THEREOF. Applicant: Icahn School of Medicine at Mount Sinai. The sequence listing filed with the application follows.

SEQUENCE LISTING (35 sequences)

SEQ ID NO: 1 - protein, 565 aa, Influenza virus A
  source 1..565: note = influenza virus A hemagglutinin subtype H1
MKANLLVLLCALAAADADTICIGYHANNSTDTVDTVLEKNVTVTHSVNLLEDSHNGKLCRLKGIAPLQLGKCNIAGWLLGNPECDPLLPVRSWSYIVETPNSENGICYPGDFIDYEELREQLSSVSSFERFEIFPKESSWPNHNTNGVTAACSHEGKSSFYRNLLWLTEKEGSYPKLKNSYVNKKGKEVLVLWGIHHPPNSKEQQNLYQNENAYVSVVTSNYNRRFTPEIAERPKVRDQAGRMNYYWTLLKPGDTIIFEANGNLIAPMYAFALSRGFGSGIITSNASMHECNTKCQTPLGAINSSLPYQNIHPVTIGECPKYVRSAKLRMVTGLRNNPSIQSRGLFGAIAGFIEGGWTGMIDGWYGYHHQNEQGSGYAADQKSTQNAINGITNKVNTVIEKMNIQFTAVGKEFNKLEKRMENLNKKVDDGFLDIWTYNAELLVLLENERTLDFHDSNVKNLYEKVKSQLKNNAKEIGNGCFEFYHKCDNECMESVRNGTYDYPKYSEESKLNREKVDGVKLESMGIYQILAIYSTVASSLVLLVSLGAISFWMCSNGSLQCRICI

SEQ ID NO: 2 - protein, 562 aa, Influenza virus A
  source 1..562: note = influenza virus A hemagglutinin subtype H2
MAIIYLILLFTAVRGDQICIGYHSNNSTEKVDTILERNVTVTHAQNILEKTHNGKLCKLNGIPPLELGDCSIAGWLLGNPECDRLLTVPEWSYIMEKENPRNGLCYPGSFNDYEELKHLLSSVTHFEKVKILPKDRWTQHTTTGGSRACAVSGNPSFFRNMVWLTKKGSNYPIAKGSYNNTSGEQMLIIWGVHHPNDETEQRTLYQNVGTYVSIGTSTLNKRSIPVIATRPKVNGQGGRMEFSWTILDIWDTINFESTGNLIAPEYGFRISKRGSSGIMKTEGTLENCETKCQTPLGAINTTLPFHNVHPLTIGECPKYVKSERLVLATGLRNVPQIESRGLFGAIAGFIEGGWQGMIDGWYGYHHSNDQGSGYAADKESTQKAIDGITNRVNSVIEKMNTQFEAVGKEFSNLEKRLENLNKKMEDGFLDVWTYNAELLVLMENERTLDFHDSNVKNLYDRVRMQLRDNAKELGNGCFEFYHKCDDECMNSVKNGTYDYPKYEEESKLNRNEIKGVKLSNMGVYQILAIYATVAGSLSLAIMIAGISLWMCSNGSLQCRICI

SEQ ID NO: 3 - protein, 566 aa, Influenza virus A
  source 1..566: note = influenza virus A hemagglutinin subtype H3
MKTIIALSYIFCLALGQDLPGNDNSTATLCLGHHAVPNGTLVKTITDDQIEVTNATELVQSSSTGKICNNPHRILDGIDCTLIDALLGDPHCDVFQNETWDLFVERSKAFSNCYPYDVPDYASLRSLVASSGTLEFITEGFTWTGVTQNGGSNACKRGPGNGFFSRLNWLTKSGSTYPVLNVTMPNNDNFDKLYIWGVHHPSTNQEQTSLYVQESGRVTVSTRRSQQSIIPNIGSRPWVRGQSSRISIYWTIVKPGDVLVINSNGNLIAPRGYFKMRTGKSSIMSSDAPIDTCISECITPNGSIPNDKPFQNVNKITYGACPKYVKQNTLKLATGMRNVPEKQTRGLFGAIAGFIENGWEGMIDGWYGFRHQNSEGTGQAADLKSTQAAIDQINGKLNRVIEKTNEKFHQIEKEFSEVEGRIQDLEKYVEDTKIDLWSYNAELLVALENQHTIDLTDSEMNKLFEKTRRQLRENAEDMGNGCFKIYHKCDNACIESIRNGTYDHDVYRDEALNNRFQIKGVELKSGYKDWILWISFAISCFLLCVVLLGFIMWACQRGNIRCNICI

SEQ ID NO: 4 - protein, 564 aa, Influenza virus A
  source 1..564: note = influenza virus A hemagglutinin subtype H4
MLSIVILFLLIAENSSQNYTGNPVICMGHHAVANGTMVKTLADDQVEVVTAQELVESQNLPELCPSPLRLVDGQTCDIINGALGSPGCDHLNGAEWDVFIERPNAVDTCYPFDVPEYQSLRSILANNGKFEFIAEEFQWNTVKQNGKSGACKRANVDDFFNRLNWLVKSDGNAYPLQNLTKINNGDYARLYIWGVHHPSTSTEQTNLYKNNPGRVTVSTKTSQTSVVPDIGSRPLVRGQSGRVSFYWTIVEPGDLIVFNTIGNLIAPRGHYKLNNQKKSTILNTAIPIGSCVSKCHTDKGSLSTTKPFQNISRIAVGDCPRYVKQGSLKLATGMRNIPEKASRGLFGAIAGFIENGWQGLIDGWYGFRHQNAEGTGTAADLKSTQAAIDQINGKLNRLIEKTNDKYHQIEKEFEQVEGRIQDLENYVEDTKIDLWSYNAELLVALENQHTIDVTDSEMNKLFERVRRQLRENAEDKGNGCFEIFHKCDNNCIESIRNGTYDHDIYRDEAINNRFQIQGVKLTQGYKDIILWISFSISCFLLVALLLAFILWACQNGNIRCQICI

SEQ ID NO: 5 - protein, 564 aa, Influenza virus A
  source 1..564: note = influenza virus A hemagglutinin subtype H5
MERIVLLLAIVSLVKSDQICIGYHANKSTKQVDTIMEKNVTVTHAQDILERTHNGKLCSLNGVKPLILRDCSVAGWLLGNPMCDEFLNLPEWLYIVEKDNPINSLCYPGDFNDYEELKYLLSSTNHFEKIRIIPRSSWSNHDASSGVSSACPYIGRSSFLRNVVWLIKKNNTYPTIKRSYNNTNQEDLLILWGIHHPNDAAEQTKLYQNPTTYVSVGTSTLNQRSIPEIATRPKVNGQSGRMEFFWTILKPNDAINFESNGNFIAPRYAYKIVKKGDSAIMKSGLAYGNCDTKCQTPVGEINSSMPFHNIHPHTIGECPKYVKSDRLVLATGLRNVPQRKKRGLFGAIAGFIEGGWQGMVDGWYGYHHSNEQGSGYAADKESTQKAIDGITNKVNSIIDKMNTRFEAVGKEFNNLERRVENLNKKMEDGFLDVWTYNVELLVLMENERTLDFHDSNVNNLYDKVRLQLKDNARELGNGCFEFYHKCDNECMESVRNGTYDYPQYSEEARLNREEISGVKLESMGVYQILSIYSTVASSLALAIMIAGLSFWMCSNGSLQCRICI

SEQ ID NO: 6 - protein, 566 aa, Influenza virus A
  source 1..566: note = influenza virus A hemagglutinin subtype H6
MIAIIVVAILATAGRSDKICIGYHANNSTTQIDTILEKNVTVTHSVELLENQKEERFCKILKKAPLDLKGCTIEGWILGNPQCDLLLGDQSWSYIVERPTAQNGICYPGVLNEVEELKALIGSGERVERFEMFPKSTWTGVDTSSGVTRACPYNSGSSFYRNLLWIIKTKSAAYSVIKGAYNNTGNQPILYFWGVHHPPDTNEQNTLYGSGDRYVRMGTESMNFAKSPEIAARPAVNGQRGRIDYYWSILKPGETLNVESNGNLIAPWYAFRFVSTSNKGAVFKSNLPIENCDATCQTVAGVLRTNKTFQNVSPLWIGECPKYVKSESLRLATGLRNVPQIETRGLFGAIAGFIEGGWTGMIDGWYGYHHENSQGSGYAADRESTQKAVDGITNKVNSIIDKMNTQFEAVDHEFSNLERRIDNLNKRMEDGFLDVWTYNAELLVLLENERTLDLHDANVKNLYERVKSQLRDNAMILGNGCFEFWHKCDDECMESVKNGTYDYPKYQDESKLNRQEIESVKLESLGVYQILAIYSTVSSSLVLVGLIIAVGLWMCSNGSMQCRICI

SEQ ID NO: 7 - protein, 563 aa, Influenza virus A
  source 1..563: note = influenza virus A hemagglutinin subtype H7
MNTQILVFALVAVIPTNADKICLGHHAVSNGTKVNTLTERGVEVVNATETVERTNIPKICSKGKRTTDLGQCGLLGTITGPPQCDQFLEFSADLIIERREGNDVCYPGKFVNEEALRQILRGSGGIDKETMGFTYSGIRTNGTTSACRRSGSSFYAEMEWLLSNTDNASFPQMTKSYKNTRRESALIVWGIHHSGSTTEQTKLYGSGNKLITVGSSKYHQSFVPSPGTRPQINGQSGRIDFHWLILDPNDTVTFSFNGAFIAPNRASFLRGKSMGIQSDVQVDANCEGECYHSGGTITSRLPFQNINSRAVGKCPRYVKQESLLLATGMKNVPEPSKKRKKRGLFGAIAGFIENGWEGLVDGWYGFRHQNAQGEGTAADYKSTQSAIDQITGKLNRLIEKTNQQFELIDNEFTEVEKQIGNLINWTKDSITEVWSYNAELIVAMENQHTIDLADSEMNRLYERVRKQLRENAEEDGTGCFEIFHKCDDDCMASIRNNTYDHSKYREEAMQNRIQIDPVKLSSGYKDVILWFSFGASCFLLLAIAMGLVFICVKNGNMRCTICI

SEQ ID NO: 8 - protein, 565 aa, Influenza virus A
  source 1..565: note = influenza virus A hemagglutinin subtype H8
MEKFIAIATLASTNAYDRICIGYQSNNSTDTVNTLIEQNVPVTQTMELVETEKHPAYCNTDLGAPLELRDCKIEAVIYGNPKCDIHLKDQGWSYIVERPSAPEGMCYPGSVENLEELRFVFSSAASYKRIRLFDYSRWNVTRSGTSKACNASTGGQSFYRSINWLTKKEPDTYDFNEGAYVNNEDGDIIFLWGIHHPPDTKEQTTLYKNANTLSSVTTNTINRSFQPNIGPRPLVRGQQGRMDYYWGILKRGETLKIRTNGNLIAPEFGYLLKGESYGRIIQNEDIPIGNCNTKCQTYAGAINSSKPFQNASRHYMGECPKYVKKASLRLAVGLRNTPSVEPRGLFGAIAGFIEGGWSGMIDGWYGFHHSNSEGTGMAADQKSTQEAIDKITNKVNNIVDKMNREFEVVNHEFSEVEKRINMINDKIDDQIEDLWAYNAELLVLLENQKTLDEHDSNVKNLFDEVKRRLSANAIDAGNGCFDILHKCDNECMETIKNGTYDHKEYEEEAKLERSKINGVKLEENTTYKILSIYSTVAASLCLAILIAGGLILGMQNGSCRCMFCI

SEQ ID NO: 9 - protein, 560 aa, Influenza virus A
  source 1..560: note = influenza virus A hemagglutinin subtype H9
METKAIIAALLMVTAANADKICIGYQSTNSTETVDTLTESNVPVTHTKELLHTEHNGMLCATDLGHPLILDTCTIEGLIYGNPSCDILLGGKEWSYIVERSSAVNGMCYPGNVENLEELRSLFSSAKSYKRIQIFPDKTWNVTYSGTSRACSNSFYRSMRWLTHKSNSYPFQNAHYTNNERENILFMWGIHHPPTDTEQTDLYKNADTTTSVTTEDINRTFKPVIGPRPLVNGQQGRIDYYWSVLKPGQTLRIRSNGNLIAPWYGHVLTGESHGRILKTDLNNGNCVVQCQTEKGGLNTTLPFHNISKYAFGNCPKYVGVKSLKLPVGLRNVPAVSSRGLFGAIAGFIEGGWPGLVAGWYGFQHSNDQGVGMAADKGSTQKAIDKITSKVNNIIDKMNKQYEVIDHEFNELEARLNMINNKIDDQIQDIWAYNAELLVLLENQKTLDEHDANVNNLYNKVKRALGSNAVEDGNGCFELYHKCDDQCMETIRNGTYDRQKYQEESRLERQKIEGVKLESEGTYKILTIYSTVASSLVLAMGFAAFLFWAMSNGSCRCNICI

SEQ ID NO: 10 - protein, 561 aa, Influenza virus A
  source 1..561: note = influenza virus A hemagglutinin subtype H10
MYKVVVIIALLGAVKGLDRICLGHHAVANGTIVKTLTNEQEEVTNATETVESTNLNKLCMKGRSYKDLGNCHPVGMLIGTPVCDPHLTGTWDTLIERENAIAHCYPGATINEEALRQKIMESGGISKMSTGFTYGSSITSAGTTKACMRNGGDSFYAELKWLVSKTKGQNFPQTTNTYRNTDTAEHLIIWGIHHPSSTQEKNDLYGTQSLSISVESSTYQNNFVPVVGARPQVNGQSGRIDFHWTLVQPGDNITFSDNGGLIAPSRVSKLTGRDLGIQSEALIDNSCESKCFWRGGSINTKLPFQNLSPRTVGQCPKYVNQRSLLLATGMRNVPEVVQGRGLFGAIAGFIENGWEGMVDGWYGFRHQNAQGTGQAADYKSTQAAIDQITGKLNRLIEKTNTEFESIESEFSETEHQIGNVINWTKDSITDIWTYNAELLVAMENQHTIDMADSEMLNLYERVRKQLRQNAEEDGKGCFEIYHTCDDSCMESIRNNTYDHSQYREEALLNRLNINPVKLSSGYKDIILWFSFGESCFVLLAVVMGLVFFCLKNGNMRCTICI

SEQ ID NO: 11 - protein, 565 aa, Influenza virus A
  source 1..565: note = influenza virus A hemagglutinin subtype H11
MEKTLLFAAIFLCVKADEICIGYLSNNSTDKVDTIIENNVTVTSSVELVETEHTGSFCSINGKQPISLGDCSFAGWILGNPMCDELIGKTSWSYIVEKPNPTNGICYPGTLESEEELRLKFSGVLEFNKFEVFTSNGWGAVNSGVGVTAACKFGGSNSFFRNMVWLIHQSGTYPVIKRTFNNTKGRDVLIVWGIHHPATLTEHQDLYKKDSSYVAVGSETYNRRFTPEINTRPRVNGQAGRMTFYWKIVKPGESITFESNGAFLAPRYAFEIVSVGNGKLFRSELNIESCSTKCQTEIGGINTNKSFHNVHRNTIGDCPKYVNVKSLKLATGPRNVPAIASRGLFGAIAGFIEGGWPGLINGWYGFQHRDEEGTGIAADKESTQKAIDQITSKVNNIVDRMNTNFESVQHEFSEIEERINQLSKHVDDSVVDIWSYNAQLLVLLENEKTLDLHDSNVRNLHEKVRRMLKDNAKDEGNGCFTFYHKCDNKCIERVRNGTYDHKEFEEESKINRQEIEGVKLDSSGNVYKILSIYSCIASSLVLAALIMGFMFWACSNGSCRCTICI

SEQ ID NO: 12 - protein, 564 aa, Influenza virus A
  source 1..564: note = influenza virus A hemagglutinin subtype H12
MEKFIILSTVLAASFAYDKICIGYQTNNSTETVNTLSEQNVPVTQVEELVHRGIDPILCGTELGSPLVLDDCSLEGLILGNPKCDLYLNGREWSYIVERPKEMEGVCYPGSIENQEELRSLFSSIKKYERVKMFDFTKWNVTYTGTSKACNNTSNQGSFYRSMRWLTLKSGQFPVQTDEYKNTRDSDIVFTWAIHHPPTSDEQVKLYKNPDTLSSVTTVEINRSFKPNIGPRPLVRGQQGRMDYYWAVLKPGQTVKIQTNGNLIAPEYGHLITGKSHGRILKNNLPMGQCVTECQLNEGVMNTSKPFQNTSKHYIGKCPKYIPSGSLKLAIGLRNVPQVQDRGLFGAIAGFIEGGWPGLVAGWYGFQHQNAEGTGIAADRDSTQRAIDNMQNKLNNVIDKMNKQFEVVNHEFSEVESRINMINSKIDDQITDIWAYNAELLVLLENQKTLDEHDANVRNLHDRVRRVLRENAIDTGDGCFEILHKCDNNCMDTIRNGTYNHKEYEEESKIERQKVNGVKLEENSTYKILSIYSSVASSLVLLLMIIGGFIFGCQNGNVRCTFCI

SEQ ID NO: 13 - protein, 566 aa, Influenza virus A
  source 1..566: note = influenza virus A hemagglutinin subtype H13
MALNVIATLTLISVCVHADRICVGYLSTNSSERVDTLLENGVPVTSSIDLIETNHTGTYCSLNGVSPVHLGDCSFEGWIVGNPACTSNFGIREWSYLIEDPAAPHGLCYPGELNNNGELRHLFSGIRSFSRTELIPPTSWGEVLDGTTSACRDNTGTNSFYRNLVWFIKKNTRYPVISKTYNNTTGRDVLVLWGIHHPVSVDETKTLYVNSDPYTLVSTKSWSEKYKLETGVRPGYNGQRSWMKIYWSLIHPGEMITFESNGGFLAPRYGYIIEEYGKGRIFQSRIRMSRCNTKCQTSVGGINTNRTFQNIDKNALGDCPKYIKSGQLKLATGLRNVPAISNRGLFGAIAGFIEGGWPGLINGWYGFQHQNEQGTGIAADKESTQKAIDQITTKINNIIDKMNGNYDSIRGEFNQVEKRINMLADRIDDAVTDIWSYNAKLLVLLENDKTLDMHDANVKNLHEQVRRELKDNAIDEGNGCFELLHKCNDSCMETIRNGTYDHTEYAEESKLKRQEIDGIKLKSEDNVYKALSIYSCIASSVVLVGLILSFIMWACSSGNCRFNVCI

SEQ ID NO: 14 - protein, 568 aa, Influenza virus A
  source 1..568: note = influenza virus A hemagglutinin subtype H14
MIALILVALALSHTAYSQITNGTTGNPIICLGHHAVENGTSVKTLTDNHVEVVSAKELVETNHTDELCPSPLKLVDGQDCHLINGALGSPGCDRLQDTTWDVFIERPTAVDTCYPFDVPDYQSLRSILASSGSLEFIAEQFTWNGVKVDGSSSACLRGGRNSFFSRLNWLTKATNGNYGPINVTKENTGSYVRLYLWGVHHPSSDNEQTDLYKVATGRVTVSTRSDQISIVPNIGSRPRVRNQSGRISIYWTLVNPGDSIIFNSIGNLIAPRGHYKISKSTKSTVLKSDKRIGSCTSPCLTDKGSIQSDKPFQNVSRIAIGNCPKYVKQGSLMLATGMRNIPGKQAKGLFGAIAGFIENGWQGLIDGWYGFRHQNAEGTGTAADLKSTQAAIDQINGKLNRLIEKTNEKYHQIEKEFEQVEGRIQDLEKYVEDTKIDLWSYNAELLVALENQHTIDVTDSEMNKLFERVRRQLRENAEDQGNGCFEIFHQCDNNCIESIRNGTYDHNIYRDEAINNRIKINPVTLTMGYKDIILWISFSMSCFVFVALILGFVLWACQNGNIRCQICI

SEQ ID NO: 15 - protein, 570 aa, Influenza virus A
  source 1..570: note = influenza virus A hemagglutinin subtype H15
MNTQIIVILVLGLSMVKSDKICLGHHAVANGTKVNTLTERGVEVVNATETVEITGIDKVCTKGKKAVDLGSCGILGTIIGPPQCDLHLEFKADLIIERRNSSDICYPGRFTNEEALRQIIRESGGIDKESMGFRYSGIRTDGATSACKRTVSSFYSEMKWLSSSMNNQVFPQLNQTYRNTRKEPALIVWGVHHSSSLDEQNKLYGTGNKLITVGSSKYQQSFSPSPGARPKVNGQAGRIDFHWMLLDPGDTVTFTFNGAFIAPDRATFLRSNAPSGIEYNGKSLGIQSDAQIDESCEGECFYSGGTINSPLPFQNIDSRAVGKCPRYVKQSSLPLALGMKNVPEKIRTRGLFGAIAGFIENGWEGLIDGWYGFRHQNAQGQGTAADYKSTQAAIDQITGKLNRLIEKTNKQFELIDNEFTEVEQQIGNVINWTRDSLTEIWSYNAELLVAMENQHTIDLADSEMNKLYERVRRQLRENAEEDGTGCFEIFHRCDDQCMESIRNNTYNHTEYRQEALQNRIMINPVKLSSGYKDVILWFSFGASCVMLLAIAMGLIFMCVKNGNLRCTICI

SEQ ID NO: 16 - protein, 565 aa, Influenza virus A
  source 1..565: note = influenza virus A hemagglutinin subtype H16
MMIKVLYFLIIVLGRYSKADKICIGYLSNNSSDTVDTLTENGVPVTSSVDLVETNHTGTYCSLNGISPIHLGDCSFEGWIVGNPSCATNINIREWSYLIEDPNAPNKFCYPGELDNNGELRHLFSGVNSFSRTELINPSKWGNVLDGVTASCLDRGASSFYRNLVWIVKKDEKYPVIKGDYNNTTGRDVLVLWGIHHPDTETTATNLYVNKNPYTLVSTKEWSKRYELEIGTRIGDGQRSWMKLYWHLMHPGERIMFESNGGLIAPRYGYIIEKYGTGRIFQSGVRMARCNTKCQTSLGGINTNKTFQNIERNALGDCPKYIKSGQLKLATGLRNVPSIGERGLFGAIAGFIEGGWPGLINGWYGFQHQNEQGTGIAADKASTQKAINEITTKINNIIEKMNGNYDSIRGEFNQVEKRINMLADRVDDAVTDIWSYNAKLLVLLENDRTLDLHDANVRNLHDQVKRALKSNAIDEGDGCFNLLHKCNDSCMETIRNGTYNHEDYREESQLKRQEIEGIKLKTEDNVYKVLSIYSCIASSIVLVGLILAFIMWACSNGSCRFNVCI

SEQ ID NO: 17 - protein, 6 aa, synthetic construct
  source 1..6: note = synthetic peptide - His tag
HHHHHH

SEQ ID NO: 18 - protein, 29 aa, synthetic construct
  REGION 1..29: note = synthetic peptide - an example of folden (trimerization) domain
GSGYIPEAPRDGQAYVRKDGEWVLLSTFL

SEQ ID NO: 19 - protein, 7 aa, synthetic construct
  source 1..7: note = synthetic peptide - an example of thrombin cleavage site
LVPRGSP

SEQ ID NO: 20 - protein, 7 aa, synthetic construct
  SITE 7: note = misc_feature - Xaa = Gly or Ser
  source 1..7: note = synthetic peptide - cleavage site recognized by Tobacco Etch Virus (TEV) protease
ENLYFQX

SEQ ID NO: 21 - protein, 568 aa, synthetic construct
  source 1..568: note = exemplary chimeric influenza virus hemagglutinin polypeptide
MKAIIVLLMVVTSNADRICTGITSSNSPHVVKTATQGEVNVTGVIPLTTTPTKSYFACDLDGVKPLILRDCSVAGWLLGNPMCDEFINVPEWSYIVEKANPVNDLCYPGDFNDYEELKHLLSRINHFEKIQIIPKSSWSSHEASLGVSSACPYQGKSSFFRNVVWLIKKNSTYPTIKRSYNNTNQEDLLVLWGIHHPNDAAEQTKLYQNPTTYISVGTSTLNQRLVPRIATRSKVNGQSGRMEFFWTILKPNDAINFESNGNFIAPEYAYKIVKKGDSTIMKSELEYGNCADCLHEKYGGLNKSKPYYTGEHAKAIGNCPIWVKTPLKLANGTKYRPPAKLLKERGFFGAIAGFLEGGWEGMIAGWHGYTSHGAHGVAVAADLKSTQEAINKITKNLNSLSELEVKNLQRLSGAMDELHNEILELDEKVDDLRADTISSQIELAVLLSNEGIINSEDEHLLALERKLKKMLGPSAVEIGNGCFETKHKCNQTCLDRIAAGTFNAGEFSLPTFDSLNITAASLNDDGLDNHTILLYYSTAASSLAVTLMLAIFIVYMVSRDNVSCSICL

SEQ ID NO: 22 - protein, 5 aa, synthetic construct
  source 1..5: note = synthetic peptide - HA1 N-terminal stem segment
DRICT

SEQ ID NO: 23 - protein, 52 aa, synthetic construct
  source 1..52: note = N-terminal sequence of hemagglutinin protein of A/Hong Kong/1/1968 (H3)
QDLPGNDNSTATLCLGHHAVPNGTLVKTITDDQIEVTNATELVQSSSTGKIC

SEQ ID NO: 24 - protein, 52 aa, synthetic construct
  source 1..52: note = N-terminal sequence of hemagglutinin protein of A/Perth/16/2009 (H3)
QKLPGNDNSTATLCLGHHAVPNGTIVKTITNDQIEVTNATELVQSSSTGEIC

SEQ ID NO: 25 - protein, 42 aa, synthetic construct
  source 1..42: note = N-terminal sequence of hemagglutinin protein of A/PR/8/34 (H1)
DTICIGYHANNSTDTVDTVLEKNVTVTHSVNLLEDSHNGKLC

SEQ ID NO: 26 - protein, 42 aa, synthetic construct
  source 1..42: note = N-terminal sequence of hemagglutinin protein of A/Cal/4/09 (H1)
DTLCIGYHANNSTDTVDTVLKKNVTVTHSVNLLEDKHNGKLC

SEQ ID NO: 27 - protein, 42 aa, synthetic construct
  source 1..42: note = N-terminal sequence of hemagglutinin protein of A/Viet Nam/1203/04 (H5)
DQICIGYHANNSTEQVDTIMEKNVTVTHAQDILEKKHNGKLC

SEQ ID NO: 28 - protein, 42 aa, synthetic construct
  source 1..42: note = N-terminal sequence of hemagglutinin protein of A/mallard/Alberta/24/01 (H7)
DKICLGHHAVANGTKVNTLTEKGIEVVNATETVETVNIKKIC

SEQ ID NO: 29 - protein, 274 aa, synthetic construct
  source 1..274: note = C-terminal sequence of hemagglutinin protein of A/Hong Kong/1/1968 (H3)
CISECITPNGSIPNDKPFQNVNKITYGACPKYVKQNTLKLATGMRNVPEKQTRGLFGAIAGFIENGWEGMIDGWYGFRHQNSEGTGQAADLKSTQAAIDQINGKLNRVIEKTNEKFHQIEKEFSEVEGRIQDLEKYVEDTKIDLWSYNAELLVALENQHTIDLTDSEMNKLFEKTRRQLRENAEDMGNGCFKIYHKCDNACIESIRNGTYDHDVYRDEALNNRFQIKGVELKSGYKDWILWISFAISCFLLCVVLLGFIMWACQRGNIRCNICI

SEQ ID NO: 30 - protein, 274 aa, synthetic construct
  source 1..274: note = C-terminal sequence of hemagglutinin protein of A/Perth/16/2009 (H3)
CNSECITPNGSIPNDKPFQNVNRITYGACPRYVKQNTLKLATGMRNVPEKQTRGIFGAIAGFIENGWEGMVDGWYGFRHQNSEGRGQAADLKSTQAAIDQINGKLNRLIGKTNEKFHQIEKEFSEVEGRIQDLEKYVEDTKIDLWSYNAELLVALENQHTIDLTDSEMNKLFEKTKKQLRENAEDMGNGCFKIYHKCDNACIGSIRNGTYDHDVYRDEALNNRFQIKGVELKSGYKDWILWISFAISCFLLCVALLGFIMWACQKGNIRCNICI

SEQ ID NO: 31 - protein, 275 aa, synthetic construct
  source 1..275: note = C-terminal sequence of hemagglutinin protein of A/PR/8/34 (H1)
CNTKCQTPLGAINSSLPYQNIHPVTIGECPKYVRSAKLRMVTGLRNTPSIQSRGLFGAIAGFIEGGWTGMIDGWYGYHHQNEQGSGYAADQKSTQNAINGITNKVNTVIEKMNIQFTAVGKEFNKLEKRMENLNKKVDDGFLDIWTYNAELLVLLENERTLDFHDSNVKNLYEKVKSQLKNNAKEIGNGCFEFYHKCDNECMESVRNGTYDYPKYSEESKLNREKVDGVKLESMGIYQILAIYSTVASSLVLLVSLGAISFWMCSNGSLQCRICI

SEQ ID NO: 32 - protein, 275 aa, synthetic construct
  source 1..275: note = C-terminal sequence of hemagglutinin protein of A/Cal/4/09 (H1)
CNTTCQTPKGAINTSLPFQNIHPITIGKCPKYVKSTKLRLATGLRNIPSIQSRGLFGAIAGFIEGGWTGMVDGWYGYHHQNEQGSGYAADLKSTQNAIDEITNKVNSVIEKMNTQFTAVGKEFNHLEKRIENLNKKVDDGFLDIWTYNAELLVLLENERTLDYHDSNVKNLYEKVRSQLKNNAKEIGNGCFEFYHKCDNTCMESVKNGTYDYPKYSEEAKLNREEIDGVKLESTRIYQILAIYSTVASSLVLVVSLGAISFWMCSNGSLQCRICI

SEQ ID NO: 33 - protein, 275 aa, synthetic construct
  source 1..275: note = C-terminal sequence of hemagglutinin protein of A/Viet Nam/1203/04 (H5)
CNTKCQTPMGAINSSMPFHNIHPLTIGECPKYVKSNRLVLATGLRNSPQRETRGLFGAIAGFIEGGWQGMVDGWYGYHHSNEQGSGYAADKESTQKAIDGVTNKVNSIIDKMNTQFEAVGREFNNLERRIENLNKKMEDGFLDVWTYNAELLVLMENERTLDFHDSNVKNLYDKVRLQLRDNAKELGNGCFEFYHKCDNECMESVRNGTYDYPQYSEEARLKREEISGVKLESIGIYQILSIYSTVASSLALAIMVAGLSLWMCSNGSLQCRICI

SEQ ID NO: 34 - protein, 275 aa, synthetic construct
  source 1..275: note = C-terminal sequence of hemagglutinin protein of A/mallard/Alberta/24/01 (H7)
CEGDCFHSGGTIVSSLPFQNINPRTVGKCPRYVKQTSLLLATGMRNVPENPKTRGLFGAIAGFIENGWEGLIDGWYGFRHQNAQGEGTAADYKSTQSAIDQITGKLNRLIDKTNQQFELIDNEFSEIEQQIGNVINWTRDSMTEVWSYNAELLVAMENQHTIDLANSEMNKLYERVRKQLRENAEEDGTGCFEIFHKCDDQCMESIRNNTYDHTQYRTESLQNRIQIDPVKLSSGYKDIILWFSFGASCFILLAIAMGLVFICIKNGNMRCTICI

SEQ ID NO: 35 - protein, 564 aa, influenza virus A
  source 1..564: note = influenza virus A hemagglutinin
MELIVLLILLNPYTFVLGDRICIGYQANQNNQTVNTLLEQNVPVTGAQEILETNHNGKLCSLNGVPPLDLQSCTLAGWLLGNPNCDSLLEAEEWSYIKINESAPDDLCFPGNFENLQDLLLEMSGVQNFTKVKLFNPQSMTGVTTNNVDQTCPFEGKPSFYRNLNWIQGNSGLPFNIEIKNPTSNPLLLLWGIHNTKDAAQQRNLYGNDYSYTIFNFGEKSEEFRPEIGQRDEVKAHQDRIDYYWGSLPAQSTLRIESTGNLIAPEYGFYYKRKEGKGGLMKSKLPISDCSTKCQTPLGALNSTLPFQNVHQQTIGNCPKYVKATSLMLATGLRNNPQMEGRGLFGAIAGFIEGGWQGMIDGWYGYHHENQEGSGYAADKEATQKAVDAITNKVNSIIDKMNSQFESNIKEFNRLELRIQHLSDRVDDALLDIWSYNTELLVLLENERTLDFHDANVKNLFEKVKAQLKDNAIDEGNGCFLLLHKCNNSCMDDIKNGTYKYMDYREESHIEKQKIDGVKLTDYSRYYIMTLYSTIASSVVLGSLIIAAFLWGCQKGSIQCKICI